European Patent Application EP 4 400 589 A1, published July 17, 2024. Title: lactase and lactase preparation. Applicant: GODO SHUSEI CO., LTD. The sequence listing filed with the application follows.

SEQUENCE LISTING (2 sequences)

SEQ ID NO: 1 - protein, 1063 aa, Bifidobacterium longum
MQHPIPTTIASSDWLTDPTVFAVNREPAHSDHRFYDHVPQPNETMSLKQNLDGLWNVAVTTAPVFGFPMNDSGNAESPDFTATDYDDTGFSRIAVPSTLETKGLLNHKYVNVQYPWDGHSDPKAPNIPTDGHVAIYRRTFETSTPVSAAIENKRRITLTFHGASTAIYVWLNGSFVGYAEDSYTPSEFDVTEALISGTNTLAVACYEYATASWLEDQDFWRMHGLFRSVELTAQPTVHIEDLHITADFEATTHAGTIDAHAVIRNIADAKQLSAALMDANGTPVWQDSYAMSDIVDTSGVPCCGTADAAIDSTAVQFRANLANIRPWSAEKPYLYTLALTVRAADNSIIEVVPQRLGFRHFEIVDGIMRLNGKRIIFRGANRHEFDARLGRAITEQEMLTDIITCKRNNINAIRTSHYPNQTRFYELCDEYGLYLIDETNLETHGSWTIPGDVETPETAIPGSNPIWEGPCVDRIASMIGRDRNHPSVLIWSLGNESYAGEVFRAMYRFAHAADSTRPVHYEGVVHDRPFDDVTDIETRMYAKPAEIEEYLTNDPKKPYISCEYMHAMGNSVGGMHLYTELERYPHYQGGFIWDFIDQALWQQLDDDTERLTYGGDWDDRPCDYEFAGDGLVFADHSPSPKLQEVKRLYAPVVLTVSDHDVTIENRNLFVSTIDFAFTAKLLADGNAIWQADYRFDVPAGETRTFPIDFPSVDAAGEITYEVDQSLATATPWAPAGYELAFGQHTVQSVVPASAGTDSTACGAVPSTADSDTSDTGTVTVGRWNIGVVSGDGRTEALLSRTQGGMVSFKRDGREMVLRRPAITCFRPLTDNDRGNGSGFDRVRWFGAGRYARIANQQFSQTETGVIAEYTYTLAEPGETQVAVRYEVDAASGRVHLAARYAGATDAPTLPAFGLEWTLPKQYENLRFYGLGPEETYRDRLHGGKLGIFERTAAEDNAPYLVPQETGNHEDVRWAEVLDAQGHGMRISQAGSEHFAASLLPYSSLMLEEATHQNELPPVRHTFLRLLAAQMGVGGDDSWGAPVHEQYQLPADRAYTLDVNLELF

SEQ ID NO: 2 - DNA, 3192 bp, Bifidobacterium longum
  source 1..3192: mol_type = genomic DNA
atgcagcatcccatccccaccaccatcgcatcatctgattggctcaccgatccgaccgtattcgccgtcaaccgcgaaccagcccattccgaccatcgcttctacgatcacgtaccgcagccgaacgaaacgatgagcctcaagcaaaaccttgacggcttgtggaatgtcgccgtgacgaccgccccggttttcggcttccccatgaacgattccggcaacgctgaatctccggatttcaccgcaaccgattatgacgacaccggtttcagccgcatcgccgttccctcaacactggaaaccaagggcttgctgaaccataagtacgtcaacgtgcagtacccctgggatggccacagcgaccccaaggctcccaacatccccactgatggtcacgtagccatttaccgccgcactttcgagacaagcacccccgtctccgccgccatcgaaaacaagcgccgcatcacgctgaccttccacggcgcctccaccgccatctacgtctggctcaacggttccttcgtcggctacgccgaggactcctacacacccagcgaattcgacgtcaccgaggcactgatttccggaaccaatacactggccgtggcctgctatgaatacgccaccgcaagttggctggaagatcaggacttttggcgcatgcacggtctgttccgctccgttgaactcaccgcgcaacccactgtgcacatcgaagacctgcacatcaccgccgatttcgaggcgaccacccatgccggcaccatcgacgcccatgccgtgatccgcaacatcgccgacgccaagcaactcagcgccgcactcatggatgccaacggcacgccggtctggcaggattcctatgccatgtccgacatcgtcgacacctccggcgtaccctgctgcggcaccgcagacgccgcgatcgacagcaccgccgtgcaattccgcgcgaatctggccaacattcgtccatggagcgccgaaaagccctacctgtacacgctggctctcaccgtgcgcgcagcagacaacagcatcatcgaagtggtgccgcaacgtctcggcttccgccatttcgaaatcgttgacggcattatgcgactcaacggcaagcgcatcatcttccgcggcgccaaccgccacgagttcgacgcgcgtttgggccgtgccatcaccgagcaggagatgctcaccgacatcatcacctgcaagcgcaacaatatcaacgctattcgcacctcccactacccgaatcagacgcgattctacgaactgtgcgatgaatacggcctgtacctgatcgacgagacgaaccttgagacccacggcagctggaccattcccggtgatgtggagacccctgaaaccgccattccgggcagcaatcccatctgggaaggcccttgcgtggaccgtatcgccagcatgatcgggcgcgaccgcaatcatccgagcgtactgatctggtctctgggtaacgaatcgtacgcaggcgaggtgttccgcgcgatgtaccgcttcgctcacgcggccgactccacgcgacccgtgcattacgaaggcgtggtgcatgaccgcccctttgacgacgtgaccgacatcgagacccgcatgtatgccaagcccgcggaaatcgaggaatatctgaccaatgatccgaagaagccctatatctcctgcgaatatatgcacgccatgggcaattcggtcggcggcatgcatctgtacaccgagctggagcgttacccgcattatcagggcggctttatctgggacttcatcgatcaggccctgtggcagcagctggacgacgacaccgaacgcctgacctacggtggcgactgggacgatcgtccctgcgactatgagttcgccggcgacggcctagtcttcgccgaccactctccctcaccgaagctgcaagaggtcaagcgtctgtacgctcccgtggtactgaccgtaagcgaccacgatgtgaccatcgaaaaccgcaatctgttcgtctccaccattgatttcgcgttcacggcgaaactgctggcggacggcaatgccatctggcaggccgactaccgctttgatgtgcccgccggcgagacccgcaccttcccgattgacttcccgtcggtggacgccgctggcgaaatcacctatgaggtcgatcagtcgctggcaacggcaacaccgtgggcaccagccggctatgaactggcgttcggccaacacaccgttcagtcagtcgtgccggcttccgccggaaccgattcgaccgcgtgcggcgcggttccctccacggctgattccgatacttccgataccggtacagtaacggttggccgctggaacatcggcgtggtcagcggtgacggacgtaccgaagcgttgctttcacgcacgcagggcggcatggtgtcattcaagcgtgacggtcgcgaaatggtgttgcgccgtccggcgatcacctgcttccgcccgctgaccgacaatgatcgcggcaatggcagcggcttcgaccgcgtgcgctggttcggtgccggccgttatgcacgtatagcgaatcagcagttctcgcaaaccgagactggtgtcatcgccgaatacacatatacgttggccgagccgggcgaaacccaagttgccgtgcgctatgaggtggatgccgccagcggacgtgtacatctggccgcccgatatgccggtgccaccgatgcgccgacgctgccggcattcggattggaatggacacttcccaagcagtacgagaacctgcgcttctacggccttggccccgaggagacctatcgcgaccgtctgcacggtggcaagctcggcattttcgagcgcaccgcggccgaagacaatgcaccgtatctggtgccgcaggagaccggcaaccatgaagacgtgcgttgggccgaagtgcttgacgcccaaggacacggcatgcgtatcagccaggccggcagcgaacatttcgcggcgagcctgttgccgtacagctcgctcatgctggaagaggcgacccaccagaacgagttgccgccggtccgtcacacgttcctgcgcctgttggccgcgcaaatgggcgtgggcggcgacgattcatggggcgcgcccgtccatgagcagtaccagctgcccgccgatcgcgcctacacgctcgacgtgaatctggaactgttctaa